European Patent Specification EP 3 070 168 B1, published July 31, 2024. Title: ANTIGEN BINDING MOLECULES COMPRISING MODIFIED ANTIBODY VARIABLE REGIONS. Applicant: CHUGAI SEIYAKU KABUSHIKI KAISHA. The sequence listing filed with the application follows.

SEQUENCE LISTING (93 sequences)

SEQ ID NO: 1 - protein, 330 aa, Homo sapiens [sequence omitted]

SEQ ID NO: 2 - protein, 326 aa, Homo sapiens
ASTKGPSVFPLAPCSRSTSESTAALGCLVKDYFPEPVTVSWNSGALTSGVHTFPAVLQSSGLYSLSSVVTVPSSNFGTQTYTCNVDHKPSNTKVDKTVERKCCVECPPCPAPPVAGPSVFLFPPKPKDTLMISRTPEVTCVVVDVSHEDPEVQFNWYVDGVEVHNAKTKPREEQFNSTFRVVSVLTVVHQDWLNGKEYKCKVSNKGLPAPIEKTISKTKGQPREPQVYTLPPSREEMTKNQVSLTCLVKGFYPSDIAVEWESNGQPENNYKTTPPMLDSDGSFFLYSKLTVDKSRWQQGNVFSCSVMHEALHNHYTQKSLSLSPGK

SEQ ID NO: 3 - protein, 377 aa, Homo sapiens
ASTKGPSVFPLAPCSRSTSGGTAALGCLVKDYFPEPVTVSWNSGALTSGVHTFPAVLQSSGLYSLSSVVTVPSSSLGTQTYTCNVNHKPSNTKVDKRVELKTPLGDTTHTCPRCPEPKSCDTPPPCPRCPEPKSCDTPPPCPRCPEPKSCDTPPPCPRCPAPELLGGPSVFLFPPKPKDTLMISRTPEVTCVVVDVSHEDPEVQFKWYVDGVEVHNAKTKPREEQYNSTFRVVSVLTVLHQDWLNGKEYKCKVSNKALPAPIEKTISKTKGQPREPQVYTLPPSREEMTKNQVSLTCLVKGFYPSDIAVEWESSGQPENNYNTTPPMLDSDGSFFLYSKLTVDKSRWQQGNIFSCSVMHEALHNRFTQKSLSLSPGK

SEQ ID NO: 4 - protein, 327 aa, Homo sapiens
ASTKGPSVFPLAPCSRSTSESTAALGCLVKDYFPEPVTVSWNSGALTSGVHTFPAVLQSSGLYSLSSVVTVPSSSLGTKTYTCNVDHKPSNTKVDKRVESKYGPPCPSCPAPEFLGGPSVFLFPPKPKDTLMISRTPEVTCVVVDVSQEDPEVQFNWYVDGVEVHNAKTKPREEQFNSTYRVVSVLTVLHQDWLNGKEYKCKVSNKGLPSSIEKTISKAKGQPREPQVYTLPPSQEEMTKNQVSLTCLVKGFYPSDIAVEWESNGQPENNYKTTPPVLDSDGSFFLYSRLTVDKSRWQEGNVFSCSVMHEALHNHYTQKSLSLSLGK

SEQ ID NO: 5 - protein, 4 aa, Artificial sequence
  An artificially synthesized peptide sequence
GGGS

SEQ ID NO: 6 - protein, 4 aa, Artificial sequence
  An artificially synthesized peptide sequence
SGGG

SEQ ID NO: 7 - protein, 5 aa, Artificial sequence
  An artificially synthesized peptide sequence
GGGGS

SEQ ID NO: 8 - protein, 5 aa, Artificial sequence
  An artificially synthesized peptide sequence
SGGGG

SEQ ID NO: 9 - protein, 6 aa, Artificial sequence
  An artificially synthesized peptide sequence
GGGGGS

SEQ ID NO: 10 - protein, 6 aa, Artificial sequence
  An artificially synthesized peptide sequence
SGGGGG

SEQ ID NO: 11 - protein, 7 aa, Artificial sequence
  An artificially synthesized peptide sequence
GGGGGGS

SEQ ID NO: 12 - protein, 7 aa, Artificial sequence
  An artificially synthesized peptide sequence
SGGGGGG

SEQ ID NO: 13 - protein, 122 aa, Rattus norvegicus
EVQLVETGGSLVQPGKSLKLTCATSGFTFSNAWMHWVRQSPEKQLEWVAQIKAKSNNYATYYAESVKGRFTISRDDSKSNIYLQMNSLKEEDTAVYYCRYVHYGAYYGVDAWGQGTSVTVSS

SEQ ID NO: 14 - protein, 112 aa, Rattus norvegicus
DVVMTQTPVSMSVSLGGQVSISCRSSQSLVHNNGNTYVSWYIQKPSQSPQLLIYKVSNRFSGISDRFSGSGSGTDFTLKISRVEPDDLGVYYCGQGTQDPYTFGAGTKLELK

SEQ ID NO: 15 - protein, 119 aa, Mus musculus
QVQLKQSGPGLVQPSQSLSITCTVSGFSLTNYGVHWVRQSPGKGLEWLGVIWSGGNTDYNTPFTSRLSINKDNSKSQVFFKMNSLQSNDTAIYYCARALTYYDYEFAYWGQGTLVTVSA

SEQ ID NO: 16 - protein, 107 aa, Mus musculus
DILLTQSPVILSVSPGERVSFSCRASQSIGTNIHWYQQRTNGSPRLLIKYASESISGIPSRFSGSGSGTDFTLSINSVESEDIADYYCQQNNNWPTTFGAGTKLELK

SEQ ID NO: 17 - protein, 447 aa, Artificial sequence
  An artificially synthesized peptide sequence
QVQLKQSGPGLVQPSQSLSITCTVSGFSLTNYGVHWVRQSPGKGLEWLGVIWSGGNTDYNTPFTSRLSINKDNSKSQVFFKMNSLQSNDTAIYYCARALTYYDYEFAYWGQGTLVTVSAASTKGPSVFPLAPSSKSTSGGTAALGCLVKDYFPEPVTVSWNSGALTSGVHTFPAVLQSSGLYSLSSVVTVPSSSLGTQTYICNVNHKPSNTKVDKKVEPKSCDKTHTCPPCPAPELLGGPSVFLFPPKPKDTLMISRTPEVTCVVVDVSHEDPEVKFNWYVDGVEVHNAKTKPREEQYNSTYRVVSVLTVLHQDWLNGKEYKCKVSNKALPAPIEKTISKAKGQPREPQVYTLPPSRDELTKNQVSLTCLVKGFYPSDIAVEWESNGQPENNYKTTPPVLDSDGSFFLYSKLTVDKSRWQQGNVFSCSVMHEALHNHYTQKSLSLSP

SEQ ID NO: 18 - protein, 447 aa, Artificial sequence
  An artificially synthesized peptide sequence
QVQLKQSGPGLVQPSQSLSITCTVSGFSLTNYGVHWVRQSPGKGLEWLGVIWSGGNTDYNTPFTSRLSINKDNSKSQVFFKMNSLQSNDTAIYYCARALTYYDYEFAYWGQGTLVTVSAASTKGPSVFPLAPSSKSTSGGTAALGCLVKDYFPEPVTVSWNSGALTSGVHTFPAVLQSSGLYSLSSVVTVPSSSLGTQTYICNVNHKPSNTKVDKKVEPKSCDKTHTCPPCPAPELLGGPSVFLFPPKPKDTLMISRTPEVTCVVVDVSHEDPEVKFNWYVDGVEVHNAKTKPREEQYNSTYRVVSVLTVLHQDWLNGKEYKCKVSNKALPAPIEKTISKAKGQPREPQVYTLPPSRKELTKNQVSLTCLVKGFYPSDIAVEWESNGQPENNYKTTPPVLDSDGSFFLYSKLTVDKSRWQQGNVFSCSVMHEALHNRYTQKSLSLSP

SEQ ID NO: 19 - protein, 447 aa, Artificial sequence
  An artificially synthesized peptide sequence
QVQLKQSGPGLVQPSQSLSITCTVSGFSLTNYGVHWVRQSPGKGLEWLGVIWSGGNTDYNTPFTSRLSINKDNSKSQVFFKMNSLQSNDTAIYYCARALTYYDYEFAYWGQGTLVTVSAASTKGPSVFPLAPSSKSTSGGTAALGCLVKDYFPEPVTVSWNSGALTSGVHTFPAVLQSSGLYSLSSVVTVPSSSLGTQTYICNVNHKPSNTKVDKKVEPKSCDKTHTCPPCPAPELLGGPSVFLFPPKPKDTLMISRTPEVTCVVVDVSHEDPEVKFNWYVDGVEVHNAKTKPREEQYNSTYRVVSVLTVLHQDWLNGKEYKCKVSNKALPAPIEKTISKAKGQPREPQVYTLPPSRDELTKNQVSLTCLVKGFYPSDIAVEWESNGQPENNYKTTPPVLDSDGSFFLYSKLTVDKSRWQQGNVFSCSVMHEALHNHYTQESLSLSP

SEQ ID NO: 20 - protein, 445 aa, Artificial sequence
  An artificially synthesized peptide sequence
DILLTQSPVILSVSPGERVSFSCRASQSIGTNIHWYQQRTNGSPRLLIKYASESISGIPSRFSGSGSGTDFTLSINSVESEDIADYYCQQNNNWPTTFGAGTKLELKSSASTKGPSVFPLAPSSKSTSGGTAALGCLVKDYFPEPVTVSWNSGALTSGVHTFPAVLQSSGLYSLSSVVTVPSSSLGTQTYICNVNHKPSNTKVDKKVEPKSCDKTHTCPPCPAPEAAGGPSVFLFPPKPKDTLMISRTPEVTCVVVDVSHEDPEVKFNWYVDGVEVHNAKTKPREEQYASTYRVVSVLTVLHQDWLNGKEYKCKVSNKALPAPIEKTISKAKGQPREPQVCTLPPSRDELTKNQVSLWCLVKGFYPSDIAVEWESNGQPENNYKTTPPVLDSDGSFFLYSKLTVDKSRWQQGNVFSCSVMHEALHNRYTQKSLSLSPHHHHHHHH

SEQ ID NO: 21 - protein, 226 aa, Artificial sequence
  An artificially synthesized peptide sequence
QVQLKQSGPGLVQPSQSLSITCTVSGFSLTNYGVHWVRQSPGKGLEWLGVIWSGGNTDYNTPFTSRLSINKDNSKSQVFFKMNSLQSNDTAIYYCARALTYYDYEFAYWGQGTLVTVSARTVAAPSVFIFPPSDEQLKSGTASVVCLLNNFYPREAKVQWKVDNALQSGNSQESVTEQDSKDSTYSLSSTLTLSKADYEKHKVYACEVTHQGLSSPVTKSFNRGEC

SEQ ID NO: 22 - protein, 458 aa, Artificial sequence
  An artificially synthesized peptide sequence
EVQLVETGGSLVQPGKSLKLTCATSGFTFSNAWMHWVRQSPEKQLEWVAQIKAKSNNYATYYAESVKGRFTISRDDSKSNIYLQMNSLKEEDTAVYYCRYVHYGAYYGVDAWGQGTSVTVSSASTKGPSVFPLAPSSKSTSGGTAALGCLVKDYFPEPVTVSWNSGALTSGVHTFPAVLQSSGLYSLSSVVTVPSSSLGTQTYICNVNHKPSNTKVDKKVEPKSCDKTHTCPPCPAPEAAGGPSVFLFPPKPKDTLMISRTPEVTCVVVDVSHEDPEVKFNWYVDGVEVHNAKTKPREEQYASTYRVVSVLTVLHQDWLNGKEYKCKVSNKALPAPIEKTISKAKGQPREPQVYTLPPSRCELTKNQVSLSCAVKGFYPSDIAVEWESNGQPENNYKTTPPVLDSDGSFFLVSKLTVDKSRWQQGNVFSCSVMHEALHNHYTQKSLSLSPDYKDDDDK

SEQ ID NO: 23 - protein, 219 aa, Artificial sequence
  An artificially synthesized peptide sequence
DVVMTQTPVSMSVSLGGQVSISCRSSQSLVHNNGNTYVSWYIQKPSQSPQLLIYKVSNRFSGISDRFSGSGSGTDFTLKISRVEPDDLGVYYCGQGTQDPYTFGAGTKLELKRTVAAPSVFIFPPSDEQLKSGTASVVCLLNNFYPREAKVQWKVDNALQSGNSQESVTEQDSKDSTYSLSSTLTLSKADYEKHKVYACEVTHQGLSSPVTKSFNRGEC

SEQ ID NO: 24 - protein, 462 aa, Artificial sequence
  An artificially synthesized peptide sequence
EVQLVETGGSLVQPGKSLKLTCATSGFTFSNAWMHWVRQSPEKQLEWVAQIKAGCRGDCLNYATYYAESVKGRFTISRDDSKSNIYLQMNSLKEEDTAVYYCRYVHYGAYYGVDAWGQGTSVTVSSASTKGPSVFPLAPSSKSTSGGTAALGCLVKDYFPEPVTVSWNSGALTSGVHTFPAVLQSSGLYSLSSVVTVPSSSLGTQTYICNVNHKPSNTKVDKKVEPKSCDKTHTCPPCPAPEAAGGPSVFLFPPKPKDTLMISRTPEVTCVVVDVSHEDPEVKFNWYVDGVEVHNAKTKPREEQYASTYRVVSVLTVLHQDWLNGKEYKCKVSNKALPAPIEKTISKAKGQPREPQVYTLPPSRCELTKNQVSLSCAVKGFYPSDIAVEWESNGQPENNYKTTPPVLDSDGSFFLVSKLTVDKSRWQQGNVFSCSVMHEALHNHYTQKSLSLSPDYKDDDDK

SEQ ID NO: 25 - protein, 462 aa, Artificial sequence
  An artificially synthesized peptide sequence
EVQLVETGGSLVQPGKSLKLTCATSGFTFSNAWMHWVRQSPEKQLEWVAQIKAKGCRGDCLYATYYAESVKGRFTISRDDSKSNIYLQMNSLKEEDTAVYYCRYVHYGAYYGVDAWGQGTSVTVSSASTKGPSVFPLAPSSKSTSGGTAALGCLVKDYFPEPVTVSWNSGALTSGVHTFPAVLQSSGLYSLSSVVTVPSSSLGTQTYICNVNHKPSNTKVDKKVEPKSCDKTHTCPPCPAPEAAGGPSVFLFPPKPKDTLMISRTPEVTCVVVDVSHEDPEVKFNWYVDGVEVHNAKTKPREEQYASTYRVVSVLTVLHQDWLNGKEYKCKVSNKALPAPIEKTISKAKGQPREPQVYTLPPSRCELTKNQVSLSCAVKGFYPSDIAVEWESNGQPENNYKTTPPVLDSDGSFFLVSKLTVDKSRWQQGNVFSCSVMHEALHNHYTQKSLSLSPDYKDDDDK

SEQ ID NO: 26 - protein, 465 aa, Artificial sequence
  An artificially synthesized peptide sequence
EVQLVETGGSLVQPGKSLKLTCATSGFTFSNAWMHWVRQSPEKQLEWVAQIKAGCRGDCLKSNNYATYYAESVKGRFTISRDDSKSNIYLQMNSLKEEDTAVYYCRYVHYGAYYGVDAWGQGTSVTVSSASTKGPSVFPLAPSSKSTSGGTAALGCLVKDYFPEPVTVSWNSGALTSGVHTFPAVLQSSGLYSLSSVVTVPSSSLGTQTYICNVNHKPSNTKVDKKVEPKSCDKTHTCPPCPAPEAAGGPSVFLFPPKPKDTLMISRTPEVTCVVVDVSHEDPEVKFNWYVDGVEVHNAKTKPREEQYASTYRVVSVLTVLHQDWLNGKEYKCKVSNKALPAPIEKTISKAKGQPREPQVYTLPPSRCELTKNQVSLSCAVKGFYPSDIAVEWESNGQPENNYKTTPPVLDSDGSFFLVSKLTVDKSRWQQGNVFSCSVMHEALHNHYTQKSLSLSPDYKDDDDK

SEQ ID NO: 27 - protein, 465 aa, Artificial sequence
  An artificially synthesized peptide sequence
EVQLVETGGSLVQPGKSLKLTCATSGFTFSNAWMHWVRQSPEKQLEWVAQIKAKGCRGDCLSNNYATYYAESVKGRFTISRDDSKSNIYLQMNSLKEEDTAVYYCRYVHYGAYYGVDAWGQGTSVTVSSASTKGPSVFPLAPSSKSTSGGTAALGCLVKDYFPEPVTVSWNSGALTSGVHTFPAVLQSSGLYSLSSVVTVPSSSLGTQTYICNVNHKPSNTKVDKKVEPKSCDKTHTCPPCPAPEAAGGPSVFLFPPKPKDTLMISRTPEVTCVVVDVSHEDPEVKFNWYVDGVEVHNAKTKPREEQYASTYRVVSVLTVLHQDWLNGKEYKCKVSNKALPAPIEKTISKAKGQPREPQVYTLPPSRCELTKNQVSLSCAVKGFYPSDIAVEWESNGQPENNYKTTPPVLDSDGSFFLVSKLTVDKSRWQQGNVFSCSVMHEALHNHYTQKSLSLSPDYKDDDDK

SEQ ID NO: 28 - protein, 465 aa, Artificial sequence
  An artificially synthesized peptide sequence
EVQLVETGGSLVQPGKSLKLTCATSGFTFSNAWMHWVRQSPEKQLEWVAQIKAKSNNYATYYAESVKGRFTISRDGCRGDCLDSKSNIYLQMNSLKEEDTAVYYCRYVHYGAYYGVDAWGQGTSVTVSSASTKGPSVFPLAPSSKSTSGGTAALGCLVKDYFPEPVTVSWNSGALTSGVHTFPAVLQSSGLYSLSSVVTVPSSSLGTQTYICNVNHKPSNTKVDKKVEPKSCDKTHTCPPCPAPEAAGGPSVFLFPPKPKDTLMISRTPEVTCVVVDVSHEDPEVKFNWYVDGVEVHNAKTKPREEQYASTYRVVSVLTVLHQDWLNGKEYKCKVSNKALPAPIEKTISKAKGQPREPQVYTLPPSRCELTKNQVSLSCAVKGFYPSDIAVEWESNGQPENNYKTTPPVLDSDGSFFLVSKLTVDKSRWQQGNVFSCSVMHEALHNHYTQKSLSLSPDYKDDDDK

SEQ ID NO: 29 - protein, 463 aa, Artificial sequence
  An artificially synthesized peptide sequence
EVQLVETGGSLVQPGKSLKLTCATSGFTFSNAWMHWVRQSPEKQLEWVAQIKAGCRGDCLNNYATYYAESVKGRFTISRDDSKSNIYLQMNSLKEEDTAVYYCRYVHYGAYYGVDAWGQGTSVTVSSASTKGPSVFPLAPSSKSTSGGTAALGCLVKDYFPEPVTVSWNSGALTSGVHTFPAVLQSSGLYSLSSVVTVPSSSLGTQTYICNVNHKPSNTKVDKKVEPKSCDKTHTCPPCPAPEAAGGPSVFLFPPKPKDTLMISRTPEVTCVVVDVSHEDPEVKFNWYVDGVEVHNAKTKPREEQYASTYRVVSVLTVLHQDWLNGKEYKCKVSNKALPAPIEKTISKAKGQPREPQVYTLPPSRCELTKNQVSLSCAVKGFYPSDIAVEWESNGQPENNYKTTPPVLDSDGSFFLVSKLTVDKSRWQQGNVFSCSVMHEALHNHYTQKSLSLSPDYKDDDDK

SEQ ID NO: 30 - protein, 465 aa, Artificial sequence
  An artificially synthesized peptide sequence
EVQLVETGGSLVQPGKSLKLTCATSGFTFSNAWMHWVRQSPEKQLEWVAQIKAKSNNYATYYAESVKGRFTISRDDSKSNIYLQMNSLKEEDTAVYYCRYVHYGGCRGDCLAYYGVDAWGQGTSVTVSSASTKGPSVFPLAPSSKSTSGGTAALGCLVKDYFPEPVTVSWNSGALTSGVHTFPAVLQSSGLYSLSSVVTVPSSSLGTQTYICNVNHKPSNTKVDKKVEPKSCDKTHTCPPCPAPEAAGGPSVFLFPPKPKDTLMISRTPEVTCVVVDVSHEDPEVKFNWYVDGVEVHNAKTKPREEQYASTYRVVSVLTVLHQDWLNGKEYKCKVSNKALPAPIEKTISKAKGQPREPQVYTLPPSRCELTKNQVSLSCAVKGFYPSDIAVEWESNGQPENNYKTTPPVLDSDGSFFLVSKLTVDKSRWQQGNVFSCSVMHEALHNHYTQKSLSLSPDYKDDDDK

SEQ ID NO: 31 - protein, 465 aa, Artificial sequence
  An artificially synthesized peptide sequence
EVQLVETGGSLVQPGKSLKLTCATSGFTFSNAWMHWVRQSPEKQLEWVAQIKAKSNNYATYYAESVKGRFTISRDDSKSNIYLQMNSLKEEDTAVYYCRYVHYGAGCRGDCLYYGVDAWGQGTSVTVSSASTKGPSVFPLAPSSKSTSGGTAALGCLVKDYFPEPVTVSWNSGALTSGVHTFPAVLQSSGLYSLSSVVTVPSSSLGTQTYICNVNHKPSNTKVDKKVEPKSCDKTHTCPPCPAPEAAGGPSVFLFPPKPKDTLMISRTPEVTCVVVDVSHEDPEVKFNWYVDGVEVHNAKTKPREEQYASTYRVVSVLTVLHQDWLNGKEYKCKVSNKALPAPIEKTISKAKGQPREPQVYTLPPSRCELTKNQVSLSCAVKGFYPSDIAVEWESNGQPENNYKTTPPVLDSDGSFFLVSKLTVDKSRWQQGNVFSCSVMHEALHNHYTQKSLSLSPDYKDDDDK

SEQ ID NO: 32 - protein, 465 aa, Artificial sequence
  An artificially synthesized peptide sequence
EVQLVETGGSLVQPGKSLKLTCATSGFTFSNAWMHWVRQSPEKQLEWVAQIKAKSNNYATYYAESVKGRFTISRDDSKSNIYLQMNSLKEEDTAVYYCRYVHYGAYGCRGDCLYGVDAWGQGTSVTVSSASTKGPSVFPLAPSSKSTSGGTAALGCLVKDYFPEPVTVSWNSGALTSGVHTFPAVLQSSGLYSLSSVVTVPSSSLGTQTYICNVNHKPSNTKVDKKVEPKSCDKTHTCPPCPAPEAAGGPSVFLFPPKPKDTLMISRTPEVTCVVVDVSHEDPEVKFNWYVDGVEVHNAKTKPREEQYASTYRVVSVLTVLHQDWLNGKEYKCKVSNKALPAPIEKTISKAKGQPREPQVYTLPPSRCELTKNQVSLSCAVKGFYPSDIAVEWESNGQPENNYKTTPPVLDSDGSFFLVSKLTVDKSRWQQGNVFSCSVMHEALHNHYTQKSLSLSPDYKDDDDK

SEQ ID NO: 33 - protein, 444 aa, Artificial sequence
  An artificially synthesized peptide sequence
QDQLVQSGAEVKKPGASVKVSCKASGFNIKDTYIQWVRQAPGQGLEWMGRIDPLRKQTKYREKFEGRVTITADTSTNTAYMELSSLRSEDTAVYYCVRSGREFDYWGQGTLVTVSSASTKGPSVFPLAPSSKSTSGGTAALGCLVKDYFPEPVTVSWNSGALTSGVHTFPAVLQSSGLYSLSSVVTVPSSSLGTQTYICNVNHKPSNTKVDKKVEPKSCDKTHTCPPCPAPEYQWGPMVFLFPPKPKDTLMISRTPEVTCVVVDVSDEEPEVKFNWYVDGVEVHNAKTKPREEQYNATYRVVSVLTVLHQDWLNGKEYKCKVSNKALPAPIEKTISKAKGQPREPQVCTLPPSRDELTKNQVSLWCLVKGFYPSDIAVEWESNGQPENNYKTTPPVLDSDGSFFLYSKLTVDKSRWQQGNVFSCSVMHEALHNHYTQKSLSLSP

SEQ ID NO: 34 - protein, 444 aa, Artificial sequence
  An artificially synthesized peptide sequence
QDQLVQSGAEVKKPGASVKVSCKASGFNIKDTYIQWVRQAPGQGLEWMGRIDPLRKQTKYREKFEGRVTITADTSTNTAYMELSSLRSEDTAVYYCVRSGREFDYWGQGTLVTVSSASTKGPSVFPLAPSSKSTSGGTAALGCLVKDYFPEPVTVSWNSGALTSGVHTFPAVLQSSGLYSLSSVVTVPSSSLGTQTYICNVNHKPSNTKVDKKVEPKSCDKTHTCPPCPAPELLGGPSVFLFPPKPKDTLMISRTPEVTCVVVDVSHEEPEVKFNWYVDGVEVHNAKTKPREEQYNSTYRVVSVLTVLHQDWLNGKEYKCKVSNDALPMPIEETISKAKGQPREPQVYTLPPSRCELTKNQVSLSCAVKGFYPSDIAVEWESNGQPENNYKTTPPVLDSDGSFFLVSKLTVDKSRWQQGNVFSCSVMHEALHNHYTQKSLSLSP

SEQ ID NO: 35 - protein, 213 aa, Artificial sequence
  An artificially synthesized peptide sequence
DIQMTQSPSSLSASVGDRVTITCRASQDIHKYIAWYQQKPGQAPRLLIQYTSTLQPGVPSRFSGSGSGTDYTFTISSLQPEDIATYYCLQYEQLRTFGGGTKVEIKRTVAAPSVFIFPPSDEQLKSGTASVVCLLNNFYPREAKVQWKVDNALQSGNSQESVTEQDSKDSTYSLSSTLTLSKADYEKHKVYACEVTHQGLSSPVTKSFNRGEC

SEQ ID NO: 36 - protein, 22 aa, Artificial sequence
  An artificially synthesized peptide sequence
RWGYHLRDRKYKGVRSHKGVPR

SEQ ID NO: 37 - protein, 480 aa, Artificial sequence
  An artificially synthesized peptide sequence
EVQLVETGGSLVQPGKSLKLTCATSGFTFSNAWMHWVRQSPEKQLEWVAQIKAKRWGYHLRDRKYKGVRSHKGVPRSNNYATYYAESVKGRFTISRDDSKSNIYLQMNSLKEEDTAVYYCRYVHYGAYYGVDAWGQGTSVTVSSASTKGPSVFPLAPSSKSTSGGTAALGCLVKDYFPEPVTVSWNSGALTSGVHTFPAVLQSSGLYSLSSVVTVPSSSLGTQTYICNVNHKPSNTKVDKKVEPKSCDKTHTCPPCPAPEAAGGPSVFLFPPKPKDTLMISRTPEVTCVVVDVSHEDPEVKFNWYVDGVEVHNAKTKPREEQYASTYRVVSVLTVLHQDWLNGKEYKCKVSNKALPAPIEKTISKAKGQPREPQVYTLPPSRCELTKNQVSLSCAVKGFYPSDIAVEWESNGQPENNYKTTPPVLDSDGSFFLVSKLTVDKSRWQQGNVFSCSVMHEALHNHYTQKSLSLSPDYKDDDDK

SEQ ID NO: 38 - protein, 482 aa, Artificial sequence
  An artificially synthesized peptide sequence
EVQLVETGGSLVQPGKSLKLTCATSGFTFSNAWMHWVRQSPEKQLEWVAQIKAKCRWGYHLRDRKYKGVRSHKGVPRCSNNYATYYAESVKGRFTISRDDSKSNIYLQMNSLKEEDTAVYYCRYVHYGAYYGVDAWGQGTSVTVSSASTKGPSVFPLAPSSKSTSGGTAALGCLVKDYFPEPVTVSWNSGALTSGVHTFPAVLQSSGLYSLSSVVTVPSSSLGTQTYICNVNHKPSNTKVDKKVEPKSCDKTHTCPPCPAPEAAGGPSVFLFPPKPKDTLMISRTPEVTCVVVDVSHEDPEVKFNWYVDGVEVHNAKTKPREEQYASTYRVVSVLTVLHQDWLNGKEYKCKVSNKALPAPIEKTISKAKGQPREPQVYTLPPSRCELTKNQVSLSCAVKGFYPSDIAVEWESNGQPENNYKTTPPVLDSDGSFFLVSKLTVDKSRWQQGNVFSCSVMHEALHNHYTQKSLSLSPDYKDDDDK

SEQ ID NO: 39 - protein, 480 aa, Artificial sequence
  An artificially synthesized peptide sequence
EVQLVETGGSLVQPGKSLKLTCATSGFTFSNAWMHWVRQSPEKQLEWVAQIKAKSNNYATYYAESVKGRFTISRDRWGYHLRDRKYKGVRSHKGVPRDSKSNIYLQMNSLKEEDTAVYYCRYVHYGAYYGVDAWGQGTSVTVSSASTKGPSVFPLAPSSKSTSGGTAALGCLVKDYFPEPVTVSWNSGALTSGVHTFPAVLQSSGLYSLSSVVTVPSSSLGTQTYICNVNHKPSNTKVDKKVEPKSCDKTHTCPPCPAPEAAGGPSVFLFPPKPKDTLMISRTPEVTCVVVDVSHEDPEVKFNWYVDGVEVHNAKTKPREEQYASTYRVVSVLTVLHQDWLNGKEYKCKVSNKALPAPIEKTISKAKGQPREPQVYTLPPSRCELTKNQVSLSCAVKGFYPSDIAVEWESNGQPENNYKTTPPVLDSDGSFFLVSKLTVDKSRWQQGNVFSCSVMHEALHNHYTQKSLSLSPDYKDDDDK

SEQ ID NO: 40 - protein, 482 aa, Artificial sequence
  An artificially synthesized peptide sequence
EVQLVETGGSLVQPGKSLKLTCATSGFTFSNAWMHWVRQSPEKQLEWVAQIKAKSNNYATYYAESVKGRFTISRDCRWGYHLRDRKYKGVRSHKGVPRCDSKSNIYLQMNSLKEEDTAVYYCRYVHYGAYYGVDAWGQGTSVTVSSASTKGPSVFPLAPSSKSTSGGTAALGCLVKDYFPEPVTVSWNSGALTSGVHTFPAVLQSSGLYSLSSVVTVPSSSLGTQTYICNVNHKPSNTKVDKKVEPKSCDKTHTCPPCPAPEAAGGPSVFLFPPKPKDTLMISRTPEVTCVVVDVSHEDPEVKFNWYVDGVEVHNAKTKPREEQYASTYRVVSVLTVLHQDWLNGKEYKCKVSNKALPAPIEKTISKAKGQPREPQVYTLPPSRCELTKNQVSLSCAVKGFYPSDIAVEWESNGQPENNYKTTPPVLDSDGSFFLVSKLTVDKSRWQQGNVFSCSVMHEALHNHYTQKSLSLSPDYKDDDDK

SEQ ID NO: 41 - protein, 477 aa, Artificial sequence
  An artificially synthesized peptide sequence
EVQLVETGGSLVQPGKSLKLTCATSGFTFSNAWMHWVRQSPEKQLEWVAQIKAKSNNYATYYAESVKGRFTISRDDSKSNIYLQMNSLKEEDTAVYYCRYVHYGAYYGVDAWGQGTSVTVSSASTKGPSVFPLAPSSKSTSGGTAALGCLVKDYFPEPVTVSWNSGALTSGVHTFPAVLQSSGLYSLSSVVTVPSSSLGTQTYICNVNHKPSNTKVDKKVEPKSCDKTHTCPPCPAPELLGGPSVFLFPPKPKDTLMISRTPEVTCVVVDVSHEEPEVKFNWYVDGVEVHNAKTKPREEQYNSTYRVVSVLTVLHQDWLNGKEYKCKVSNDALPMPIEETISKAKGQPREPQVYTLPPSRCELTKNQVSLSCAVKGFYPSDIAVEWESNGQPENNYKTTPPVLDSDGSFFLVSKLTVDKSRWQQGNVFSCSVMHEALHNHYTQKSLSLSPGGGGSRWGYHLRDRKYKGVRSHKGVPR

SEQ ID NO: 42 - protein, 479 aa, Artificial sequence
  An artificially synthesized peptide sequence
EVQLVETGGSLVQPGKSLKLTCATSGFTFSNAWMHWVRQSPEKQLEWVAQIKAKSNNYATYYAESVKGRFTISRDDSKSNIYLQMNSLKEEDTAVYYCRYVHYGAYYGVDAWGQGTSVTVSSASTKGPSVFPLAPSSKSTSGGTAALGCLVKDYFPEPVTVSWNSGALTSGVHTFPAVLQSSGLYSLSSVVTVPSSSLGTQTYICNVNHKPSNTKVDKKVEPKSCDKTHTCPPCPAPELLGGPSVFLFPPKPKDTLMISRTPEVTCVVVDVSHEEPEVKFNWYVDGVEVHNAKTKPREEQYNSTYRVVSVLTVLHQDWLNGKEYKCKVSNDALPMPIEETISKAKGQPREPQVYTLPPSRCELTKNQVSLSCAVKGFYPSDIAVEWESNGQPENNYKTTPPVLDSDGSFFLVSKLTVDKSRWQQGNVFSCSVMHEALHNHYTQKSLSLSPGGGGSCRWGYHLRDRKYKGVRSHKGVPRC

SEQ ID NO: 43 - protein, 461 aa, Artificial sequence
  An artificially synthesized peptide sequence
EVQLVETGGSLVQPGKSLKLTCATSGFTFSNAWMHWVRQSPEKQLEWVAQIKAKGGSSNNYATYYAESVKGRFTISRDDSKSNIYLQMNSLKEEDTAVYYCRYVHYGAYYGVDAWGQGTSVTVSSASTKGPSVFPLAPSSKSTSGGTAALGCLVKDYFPEPVTVSWNSGALTSGVHTFPAVLQSSGLYSLSSVVTVPSSSLGTQTYICNVNHKPSNTKVDKKVEPKSCDKTHTCPPCPAPEAAGGPSVFLFPPKPKDTLMISRTPEVTCVVVDVSHEDPEVKFNWYVDGVEVHNAKTKPREEQYASTYRVVSVLTVLHQDWLNGKEYKCKVSNKALPAPIEKTISKAKGQPREPQVYTLPPSRCELTKNQVSLSCAVKGFYPSDIAVEWESNGQPENNYKTTPPVLDSDGSFFLVSKLTVDKSRWQQGNVFSCSVMHEALHNHYTQKSLSLSPDYKDDDDK

SEQ ID NO: 44 - protein, 464 aa, Artificial sequence
  An artificially synthesized peptide sequence
EVQLVETGGSLVQPGKSLKLTCATSGFTFSNAWMHWVRQSPEKQLEWVAQIKAKGGSGGSSNNYATYYAESVKGRFTISRDDSKSNIYLQMNSLKEEDTAVYYCRYVHYGAYYGVDAWGQGTSVTVSSASTKGPSVFPLAPSSKSTSGGTAALGCLVKDYFPEPVTVSWNSGALTSGVHTFPAVLQSSGLYSLSSVVTVPSSSLGTQTYICNVNHKPSNTKVDKKVEPKSCDKTHTCPPCPAPEAAGGPSVFLFPPKPKDTLMISRTPEVTCVVVDVSHEDPEVKFNWYVDGVEVHNAKTKPREEQYASTYRVVSVLTVLHQDWLNGKEYKCKVSNKALPAPIEKTISKAKGQPREPQVYTLPPSRCELTKNQVSLSCAVKGFYPSDIAVEWESNGQPENNYKTTPPVLDSDGSFFLVSKLTVDKSRWQQGNVFSCSVMHEALHNHYTQKSLSLSPDYKDDDDK

SEQ ID NO: 45 - protein, 467 aa, Artificial sequence
  An artificially synthesized peptide sequence
EVQLVETGGSLVQPGKSLKLTCATSGFTFSNAWMHWVRQSPEKQLEWVAQIKAKGGSGGSGGSSNNYATYYAESVKGRFTISRDDSKSNIYLQMNSLKEEDTAVYYCRYVHYGAYYGVDAWGQGTSVTVSSASTKGPSVFPLAPSSKSTSGGTAALGCLVKDYFPEPVTVSWNSGALTSGVHTFPAVLQSSGLYSLSSVVTVPSSSLGTQTYICNVNHKPSNTKVDKKVEPKSCDKTHTCPPCPAPEAAGGPSVFLFPPKPKDTLMISRTPEVTCVVVDVSHEDPEVKFNWYVDGVEVHNAKTKPREEQYASTYRVVSVLTVLHQDWLNGKEYKCKVSNKALPAPIEKTISKAKGQPREPQVYTLPPSRCELTKNQVSLSCAVKGFYPSDIAVEWESNGQPENNYKTTPPVLDSDGSFFLVSKLTVDKSRWQQGNVFSCSVMHEALHNHYTQKSLSLSPDYKDDDDK

SEQ ID NO: 46 - protein, 461 aa, Artificial sequence
  An artificially synthesized peptide sequence
EVQLVETGGSLVQPGKSLKLTCATSGFTFSNAWMHWVRQSPEKQLEWVAQIKAKSNNYATYYAESVKGRFTISRDGGSDSKSNIYLQMNSLKEEDTAVYYCRYVHYGAYYGVDAWGQGTSVTVSSASTKGPSVFPLAPSSKSTSGGTAALGCLVKDYFPEPVTVSWNSGALTSGVHTFPAVLQSSGLYSLSSVVTVPSSSLGTQTYICNVNHKPSNTKVDKKVEPKSCDKTHTCPPCPAPEAAGGPSVFLFPPKPKDTLMISRTPEVTCVVVDVSHEDPEVKFNWYVDGVEVHNAKTKPREEQYASTYRVVSVLTVLHQDWLNGKEYKCKVSNKALPAPIEKTISKAKGQPREPQVYTLPPSRCELTKNQVSLSCAVKGFYPSDIAVEWESNGQPENNYKTTPPVLDSDGSFFLVSKLTVDKSRWQQGNVFSCSVMHEALHNHYTQKSLSLSPDYKDDDDK

SEQ ID NO: 47 - protein, 464 aa, Artificial sequence
  An artificially synthesized peptide sequence
EVQLVETGGSLVQPGKSLKLTCATSGFTFSNAWMHWVRQSPEKQLEWVAQIKAKSNNYATYYAESVKGRFTISRDGGSGGSDSKSNIYLQMNSLKEEDTAVYYCRYVHYGAYYGVDAWGQGTSVTVSSASTKGPSVFPLAPSSKSTSGGTAALGCLVKDYFPEPVTVSWNSGALTSGVHTFPAVLQSSGLYSLSSVVTVPSSSLGTQTYICNVNHKPSNTKVDKKVEPKSCDKTHTCPPCPAPEAAGGPSVFLFPPKPKDTLMISRTPEVTCVVVDVSHEDPEVKFNWYVDGVEVHNAKTKPREEQYASTYRVVSVLTVLHQDWLNGKEYKCKVSNKALPAPIEKTISKAKGQPREPQVYTLPPSRCELTKNQVSLSCAVKGFYPSDIAVEWESNGQPENNYKTTPPVLDSDGSFFLVSKLTVDKSRWQQGNVFSCSVMHEALHNHYTQKSLSLSPDYKDDDDK

SEQ ID NO: 48 - protein, 467 aa, Artificial sequence
  An artificially synthesized peptide sequence
EVQLVETGGSLVQPGKSLKLTCATSGFTFSNAWMHWVRQSPEKQLEWVAQIKAKSNNYATYYAESVKGRFTISRDGGSGGSGGSDSKSNIYLQMNSLKEEDTAVYYCRYVHYGAYYGVDAWGQGTSVTVSSASTKGPSVFPLAPSSKSTSGGTAALGCLVKDYFPEPVTVSWNSGALTSGVHTFPAVLQSSGLYSLSSVVTVPSSSLGTQTYICNVNHKPSNTKVDKKVEPKSCDKTHTCPPCPAPEAAGGPSVFLFPPKPKDTLMISRTPEVTCVVVDVSHEDPEVKFNWYVDGVEVHNAKTKPREEQYASTYRVVSVLTVLHQDWLNGKEYKCKVSNKALPAPIEKTISKAKGQPREPQVYTLPPSRCELTKNQVSLSCAVKGFYPSDIAVEWESNGQPENNYKTTPPVLDSDGSFFLVSKLTVDKSRWQQGNVFSCSVMHEALHNHYTQKSLSLSPDYKDDDDK

SEQ ID NO: 49 - protein, 461 aa, Artificial sequence
  An artificially synthesized peptide sequence
EVQLVETGGSLVQPGKSLKLTCATSGFTFSNAWMHWVRQSPEKQLEWVAQIKAKSNNYATYYAESVKGRFTISRDDSKSNIYLQMNSLKEEDTAVYYCRYVHYGAGGSYYGVDAWGQGTSVTVSSASTKGPSVFPLAPSSKSTSGGTAALGCLVKDYFPEPVTVSWNSGALTSGVHTFPAVLQSSGLYSLSSVVTVPSSSLGTQTYICNVNHKPSNTKVDKKVEPKSCDKTHTCPPCPAPEAAGGPSVFLFPPKPKDTLMISRTPEVTCVVVDVSHEDPEVKFNWYVDGVEVHNAKTKPREEQYASTYRVVSVLTVLHQDWLNGKEYKCKVSNKALPAPIEKTISKAKGQPREPQVYTLPPSRCELTKNQVSLSCAVKGFYPSDIAVEWESNGQPENNYKTTPPVLDSDGSFFLVSKLTVDKSRWQQGNVFSCSVMHEALHNHYTQKSLSLSPDYKDDDDK

SEQ ID NO: 50 - protein, 464 aa, Artificial sequence
  An artificially synthesized peptide sequence
EVQLVETGGSLVQPGKSLKLTCATSGFTFSNAWMHWVRQSPEKQLEWVAQIKAKSNNYATYYAESVKGRFTISRDDSKSNIYLQMNSLKEEDTAVYYCRYVHYGAGGSGGSYYGVDAWGQGTSVTVSSASTKGPSVFPLAPSSKSTSGGTAALGCLVKDYFPEPVTVSWNSGALTSGVHTFPAVLQSSGLYSLSSVVTVPSSSLGTQTYICNVNHKPSNTKVDKKVEPKSCDKTHTCPPCPAPEAAGGPSVFLFPPKPKDTLMISRTPEVTCVVVDVSHEDPEVKFNWYVDGVEVHNAKTKPREEQYASTYRVVSVLTVLHQDWLNGKEYKCKVSNKALPAPIEKTISKAKGQPREPQVYTLPPSRCELTKNQVSLSCAVKGFYPSDIAVEWESNGQPENNYKTTPPVLDSDGSFFLVSKLTVDKSRWQQGNVFSCSVMHEALHNHYTQKSLSLSPDYKDDDDK

SEQ ID NO: 51 - protein, 467 aa, Artificial sequence
  An artificially synthesized peptide sequence
EVQLVETGGSLVQPGKSLKLTCATSGFTFSNAWMHWVRQSPEKQLEWVAQIKAKSNNYATYYAESVKGRFTISRDDSKSNIYLQMNSLKEEDTAVYYCRYVHYGAGGSGGSGGSYYGVDAWGQGTSVTVSSASTKGPSVFPLAPSSKSTSGGTAALGCLVKDYFPEPVTVSWNSGALTSGVHTFPAVLQSSGLYSLSSVVTVPSSSLGTQTYICNVNHKPSNTKVDKKVEPKSCDKTHTCPPCPAPEAAGGPSVFLFPPKPKDTLMISRTPEVTCVVVDVSHEDPEVKFNWYVDGVEVHNAKTKPREEQYASTYRVVSVLTVLHQDWLNGKEYKCKVSNKALPAPIEKTISKAKGQPREPQVYTLPPSRCELTKNQVSLSCAVKGFYPSDIAVEWESNGQPENNYKTTPPVLDSDGSFFLVSKLTVDKSRWQQGNVFSCSVMHEALHNHYTQKSLSLSPDYKDDDDK

SEQ ID NO: 52 - protein, 122 aa, Artificial sequence
  An artificially synthesized peptide sequence
QVQLVESGGGVVQPGRSLRLSCAASGFTFSNAWMHWVRQAPGKGLEWVAQIKAKSNNYATYYAESVKGRFTISRDDSKNSLYLQMNSLKTEDTAVYYCRYVHYGAYYGVDAWGQGTTVTVSS

SEQ ID NO: 53 - protein, 112 aa, Artificial sequence
  An artificially synthesized peptide sequence
DIVMTQSPLSLPVTPGEPASISCRSSQSLVHSNRNTYLHWYQQKPGQAPRLLIYKVSNRFSGVPDRFSGSGSGTDFTLKISRVEAEDVGVYYCGQGTQVPYTFGQGTKLEIK

SEQ ID NO: 54 - protein, 336 aa, Artificial sequence
  An artificially synthesized peptide sequence
ASTKGPSVFPLAPSSKSTSGGTAALGCLVKDYFPEPVTVSWNSGALTSGVHTFPAVLQSSGLYSLSSVVTVPSSSLGTQTYICNVNHKPSNTKVDKKVEPKSCDKTHTCPPCPAPEAAGGPSVFLFPPKPKDTLMISRTPEVTCVVVDVSHEDPEVKFNWYVDGVEVHNAKTKPREEQYASTYRVVSVLTVLHQDWLNGKEYKCKVSNKALPAPIEKTISKAKGQPREPQVYTLPPSRCELTKNQVSLSCAVKGFYPSDIAVEWESNGQPENNYKTTPPVLDSDGSFFLVSKLTVDKSRWQQGNVFSCSVMHEALHNHYTQKSLSLSPDYKDDDDK

SEQ ID NO: 55 - protein, 107 aa, Homo sapiens [sequence omitted]

SEQ ID NO: 56 - protein, 230 aa, Artificial sequence
  An artificially synthesized peptide sequence
EPKSSDKTHTCPPCPAPELLGGPSVFLFPPKPKDTLMISRTPEVTCVVVDVSHEDPEVKFNWYVDGVEVHNAKTKPREEQYNSTYRVVSVLTVLHQDWLNGKEYKCKVSNKALPAPIEKTISKAKGQPREPQVCTLPPSRDELTKNQVSLWCLVKGFYPSDIAVEWESNGQPENNYKTTPPVLDSDGSFFLYSKLTVDKSRWQQGNVFSCSVMHEALHNRYTQKSLSLSP

SEQ ID NO: 57 - protein, 449 aa, Artificial sequence
  An artificially synthesized peptide sequence
QVQLQESGPGLVRPSQTLSLTCTVSGYSITSDHAWSWVRQPPGRGLEWIGYISYSGITTYNPSLKSRVTMLRDTSKNQFSLRLSSVTAADTAVYYCARSLARTTAMDYWGQGSLVTVSSASTKGPSVFPLAPSSKSTSGGTAALGCLVKDYFPEPVTVSWNSGALTSGVHTFPAVLQSSGLYSLSSVVTVPSSSLGTQTYICNVNHKPSNTKVDKKVEPKSCDKTHTCPPCPAPELLGGPSVFLFPPKPKDTLMISRTPEVTCVVVDVSHEDPEVKFNWYVDGVEVHNAKTKPREEQYNSTYRVVSVLTVLHQDWLNGKEYKCKVSNKALPAPIEKTISKAKGQPREPQVYTLPPSRDELTKNQVSLTCLVKGFYPSDIAVEWESNGQPENNYKTTPPVLDSDGSFFLYSKLTVDKSRWQQGNVFSCSVMHEALHNHYTQKSLSLSPGK

SEQ ID NO: 58 - protein, 214 aa, Artificial sequence [sequence omitted]

SEQ ID NO: 59 - protein, 458 aa, Artificial sequence
  An artificially synthesized peptide sequence
QVQLVESGGGLVQPGRSLRLSCAASGFTFSNAWMHWVRQAPGKGLEWVAQIKDKSNNYATYYAESVKGRFTISRDDSKNSIYLQMNSLKTEDTAVYYCRYVHYAAYYGVDAWGQGTTVTVSSASTKGPSVFPLAPSSKSTSGGTAALGCLVKDYFPEPVTVSWNSGALTSGVHTFPAVLQSSGLYSLSSVVTVPSSSLGTQTYICNVNHKPSNTKVDKKVEPKSCDKTHTCPPCPAPEAAGGPSVFLFPPKPKDTLMISRTPEVTCVVVDVSHEDPEVKFNWYVDGVEVHNAKTKPREEQYASTYRVVSVLTVLHQDWLNGKEYKCKVSNKALPAPIEKTISKAKGQPREPQVYTLPPSRCELTKNQVSLSCAVKGFYPSDIAVEWESNGQPENNYKTTPPVLDSDGSFFLVSKLTVDKSRWQQGNVFSCSVMHEALHNHYTQKSLSLSPDYKDDDDK

SEQ ID NO: 60 - protein, 15 aa, Artificial sequence
  An artificially synthesized peptide sequence
QDGNEEMGGITQTPY

SEQ ID NO: 61 - protein, 467 aa, Artificial sequence
  An artificially synthesized peptide sequence
QVQLVESGGGLVQPGRSLRLSCAASGFTFSSAWMHWVRQAPGKGLEWVAQIKDKGNGYNAYYAPSVKGRFTISRDDSKNSIYLQMNSLKTEDTAVYYCRYVHYTTSYFGLFGGGGGGVDAWGQGTTVTVSSASTKGPSVFPLAPSSKSTSGGTAALGCLVKDYFPEPVTVSWNSGALTSGVHTFPAVLQSSGLYSLSSVVTVPSSSLGTQTYICNVNHKPSNTKVDKKVEPKSCDKTHTCPPCPAPEAAGGPSVFLFPPKPKDTLMISRTPEVTCVVVDVSHEDPEVKFNWYVDGVEVHNAKTKPREEQYASTYRVVSVLTVLHQDWLNGKEYKCKVSNKALPAPIEKTISKAKGQPREPQVYTLPPSRCELTKNQVSLSCAVKGFYPSDIAVEWESNGQPENNYKTTPPVLDSDGSFFLVSKLTVDKSRWQQGNVFSCSVMHEALHNHYTQKSLSLSPDYKDDDDK

SEQ ID NO: 62 - protein, 467 aa, Artificial sequence; identical to SEQ ID NO: 61
  An artificially synthesized peptide sequence

SEQ ID NO: 63 - protein, 464 aa, Artificial sequence
  An artificially synthesized peptide sequence
QVQLVESGGGLVQPGRSLRLSCAASGFTFSNAWMHWVRQAPGKGLEWVAQIKDKGQQYAAYYAPSVKGRFTISRDDSKNSIYLQMNSLKTEDTAVYYCRYVHYQTYSDGSFYFGVDAWGQGTTVTVSSASTKGPSVFPLAPSSKSTSGGTAALGCLVKDYFPEPVTVSWNSGALTSGVHTFPAVLQSSGLYSLSSVVTVPSSSLGTQTYICNVNHKPSNTKVDKKVEPKSCDKTHTCPPCPAPEAAGGPSVFLFPPKPKDTLMISRTPEVTCVVVDVSHEDPEVKFNWYVDGVEVHNAKTKPREEQYASTYRVVSVLTVLHQDWLNGKEYKCKVSNKALPAPIEKTISKAKGQPREPQVYTLPPSRCELTKNQVSLSCAVKGFYPSDIAVEWESNGQPENNYKTTPPVLDSDGSFFLVSKLTVDKSRWQQGNVFSCSVMHEALHNHYTQKSLSLSPDYKDDDDK

SEQ ID NO: 64 - protein, 464 aa, Artificial sequence
  An artificially synthesized peptide sequence
QVQLVESGGGLVQPGRSLRLSCAASGFTFSNAWMHWVRQAPGKGLEWVAQIKDRVNQYANYYAESVKGRFTISRDDSKNSIYLQMNSLKTEDTAVYYCRYVHYGLTGYFSGQGGVDAWGQGTTVTVSSASTKGPSVFPLAPSSKSTSGGTAALGCLVKDYFPEPVTVSWNSGALTSGVHTFPAVLQSSGLYSLSSVVTVPSSSLGTQTYICNVNHKPSNTKVDKKVEPKSCDKTHTCPPCPAPEAAGGPSVFLFPPKPKDTLMISRTPEVTCVVVDVSHEDPEVKFNWYVDGVEVHNAKTKPREEQYASTYRVVSVLTVLHQDWLNGKEYKCKVSNKALPAPIEKTISKAKGQPREPQVYTLPPSRCELTKNQVSLSCAVKGFYPSDIAVEWESNGQPENNYKTTPPVLDSDGSFFLVSKLTVDKSRWQQGNVFSCSVMHEALHNHYTQKSLSLSPDYKDDDDK

SEQ ID NO: 65 - protein, 464 aa, Artificial sequence
  An artificially synthesized peptide sequence
QVQLVESGGGLVQPGRSLRLSCAASGFTFSNAWMHWVRQAPGKGLEWVAQIKDRVNQYANYYAESVKGRLTISRDDSKNSIYLQMNSLKTEDTAVYYCRYVHYGLTGYFSGQGGVDAWGQGTTVTVSSASTKGPSVFPLAPSSKSTSGGTAALGCLVKDYFPEPVTVSWNSGALTSGVHTFPAVLQSSGLYSLSSVVTVPSSSLGTQTYICNVNHKPSNTKVDKKVEPKSCDKTHTCPPCPAPEAAGGPSVFLFPPKPKDTLMISRTPEVTCVVVDVSHEDPEVKFNWYVDGVEVHNAKTKPREEQYASTYRVVSVLTVLHQDWLNGKEYKCKVSNKALPAPIEKTISKAKGQPREPQVYTLPPSRCELTKNQVSLSCAVKGFYPSDIAVEWESNGQPENNYKTTPPVLDSDGSFFLVSKLTVDKSRWQQGNVFSCSVMHEALHNHYTQKSLSLSPDYKDDDDK

SEQ ID NO: 66 - protein, 464 aa, Artificial sequence
  An artificially synthesized peptide sequence
QVQLVESGGGLVQPGRSLRLSCAASGFAFSNAWMHWVRQAPGKGLEWVAQIKDRVNQYANYYAESVKGRFTISRDDSKNSIYLQMNSLKTEDTAVYYCRYVHYGLTGYFSGQGGVDAWGQGTTVTVSSASTKGPSVFPLAPSSKSTSGGTAALGCLVKDYFPEPVTVSWNSGALTSGVHTFPAVLQSSGLYSLSSVVTVPSSSLGTQTYICNVNHKPSNTKVDKKVEPKSCDKTHTCPPCPAPEAAGGPSVFLFPPKPKDTLMISRTPEVTCVVVDVSHEDPEVKFNWYVDGVEVHNAKTKPREEQYASTYRVVSVLTVLHQDWLNGKEYKCKVSNKALPAPIEKTISKAKGQPREPQVYTLPPSRCELTKNQVSLSCAVKGFYPSDIAVEWESNGQPENNYKTTPPVLDSDGSFFLVSKLTVDKSRWQQGNVFSCSVMHEALHNHYTQKSLSLSPDYKDDDDK

SEQ ID NO: 67 - protein, 464 aa, Artificial sequence
  An artificially synthesized peptide sequence
QVQLVESGGGLVQPGRSLRLSCAASGFTFSNAWMHWVRQAPGKGLEWVAQIKDRVNQYANYYAECVKGRFTISRDDSKNSIYLQMNSLKTEDTAVYYCRYVHYGLTGYFSGQGGVDAWGQGTTVTVSSASTKGPSVFPLAPSSKSTSGGTAALGCLVKDYFPEPVTVSWNSGALTSGVHTFPAVLQSSGLYSLSSVVTVPSSSLGTQTYICNVNHKPSNTKVDKKVEPKSCDKTHTCPPCPAPEAAGGPSVFLFPPKPKDTLMISRTPEVTCVVVDVSHEDPEVKFNWYVDGVEVHNAKTKPREEQYASTYRVVSVLTVLHQDWLNGKEYKCKVSNKALPAPIEKTISKAKGQPREPQVYTLPPSRCELTKNQVSLSCAVKGFYPSDIAVEWESNGQPENNYKTTPPVLDSDGSFFLVSKLTVDKSRWQQGNVFSCSVMHEALHNHYTQKSLSLSPDYKDDDDK

SEQ ID NO: 68 - protein, 464 aa, Artificial sequence
  An artificially synthesized peptide sequence
QVQLVESGGGLVQPGRSLRLSCAASGFTFSSAWMHWVRQAPGKGLEWVAQIKDKQNQYNAYYAESVKGRFTISRDDSKNSIYLQMNSLKTEDTAVYYCRYVHYATSDGFLPYFGVDAWGQGTTVTVSSASTKGPSVFPLAPSSKSTSGGTAALGCLVKDYFPEPVTVSWNSGALTSGVHTFPAVLQSSGLYSLSSVVTVPSSSLGTQTYICNVNHKPSNTKVDKKVEPKSCDKTHTCPPCPAPEAAGGPSVFLFPPKPKDTLMISRTPEVTCVVVDVSHEDPEVKFNWYVDGVEVHNAKTKPREEQYASTYRVVSVLTVLHQDWLNGKEYKCKVSNKALPAPIEKTISKAKGQPREPQVYTLPPSRCELTKNQVSLSCAVKGFYPSDIAVEWESNGQPENNYKTTPPVLDSDGSFFLVSKLTVDKSRWQQGNVFSCSVMHEALHNHYTQKSLSLSPDYKDDDDK

SEQ ID NO: 69 - protein, 464 aa, Artificial sequence
  An artificially synthesized peptide sequence
QVQLVESGGGLVQPGRSLRLSCAASGFTFSNAWMHWVRQAPGKGLEWVAQIKDRASGYNNYYAESVKGRFTISRDDSKNSIYLQMNSLKTEDTAVYYCRYVHYAQSVSAFFQYGVDAWGQGTTVTVSSASTKGPSVFPLAPSSKSTSGGTAALGCLVKDYFPEPVTVSWNSGALTSGVHTFPAVLQSSGLYSLSSVVTVPSSSLGTQTYICNVNHKPSNTKVDKKVEPKSCDKTHTCPPCPAPEAAGGPSVFLFPPKPKDTLMISRTPEVTCVVVDVSHEDPEVKFNWYVDGVEVHNAKTKPREEQYASTYRVVSVLTVLHQDWLNGKEYKCKVSNKALPAPIEKTISKAKGQPREPQVYTLPPSRCELTKNQVSLSCAVKGFYPSDIAVEWESNGQPENNYKTTPPVLDSDGSFFLVSKLTVDKSRWQQGNVFSCSVMHEALHNHYTQKSLSLSPDYKDDDDK

SEQ ID NO: 70 - protein, 464 aa, Artificial sequence
  An artificially synthesized peptide sequence
QVQLVESGGGLVQPGRSLRLSCAASGFTFSNAWMHWVRQAPGKGLEWVAQIKDKQSQYANYYAPSVKGRFTISRDDSKNSIYLQMNSLKTEDTAVYYCRYVHYQSTSYSFYQGGVDAWGQGTTVTVSSASTKGPSVFPLAPSSKSTSGGTAALGCLVKDYFPEPVTVSWNSGALTSGVHTFPAVLQSSGLYSLSSVVTVPSSSLGTQTYICNVNHKPSNTKVDKKVEPKSCDKTHTCPPCPAPEAAGGPSVFLFPPKPKDTLMISRTPEVTCVVVDVSHEDPEVKFNWYVDGVEVHNAKTKPREEQYASTYRVVSVLTVLHQDWLNGKEYKCKVSNKALPAPIEKTISKAKGQPREPQVYTLPPSRCELTKNQVSLSCAVKGFYPSDIAVEWESNGQPENNYKTTPPVLDSDGSFFLVSKLTVDKSRWQQGNVFSCSVMHEALHNHYTQKSLSLSPDYKDDDDK

SEQ ID NO: 71 - protein, 464 aa, Artificial sequence
  An artificially synthesized peptide sequence
QVQLVESGGGLVQPGRSLRLSCAASGFTFSNAWMHWVRQAPGKGLEWVAQIKDKQSQYANYYAPSVKGRFTISRDDSKSSIYLQMNSLKTEDTAVYYCRYVHYQSTSYSFYQGGVDAWGQGTTVTVSSASTKGPSVFPLAPSSKSTSGGTAALGCLVKDYFPEPVTVSWNSGALTSGVHTFPAVLQSSGLYSLSSVVTVPSSSLGTQTYICNVNHKPSNTKVDKKVEPKSCDKTHTCPPCPAPEAAGGPSVFLFPPKPKDTLMISRTPEVTCVVVDVSHEDPEVKFNWYVDGVEVHNAKTKPREEQYASTYRVVSVLTVLHQDWLNGKEYKCKVSNKALPAPIEKTISKAKGQPREPQVYTLPPSRCELTKNQVSLSCAVKGFYPSDIAVEWESNGQPENNYKTTPPVLDSDGSFFLVSKLTVDKSRWQQGNVFSCSVMHEALHNHYTQKSLSLSPDYKDDDDK

SEQ ID NO: 72 - protein, 464 aa, Artificial sequence
  An artificially synthesized peptide sequence
QVQLVESGGGLVQPGRSLRLSCAASGFTFSNAWMHWVRQAPGKGLEWVAQIKDRGNNYAAYYAESVKGRFTISRDDSKNSIYLQMNSLKTEDTAVYYCRYVHYGSYFFASFYFGVDIWGQGTTVTVSSASTKGPSVFPLAPSSKSTSGGTAALGCLVKDYFPEPVTVSWNSGALTSGVHTFPAVLQSSGLYSLSSVVTVPSSSLGTQTYICNVNHKPSNTKVDKKVEPKSCDKTHTCPPCPAPEAAGGPSVFLFPPKPKDTLMISRTPEVTCVVVDVSHEDPEVKFNWYVDGVEVHNAKTKPREEQYASTYRVVSVLTVLHQDWLNGKEYKCKVSNKALPAPIEKTISKAKGQPREPQVYTLPPSRCELTKNQVSLSCAVKGFYPSDIAVEWESNGQPENNYKTTPPVLDSDGSFFLVSKLTVDKSRWQQGNVFSCSVMHEALHNHYTQKSLSLSPDYKDDDDK

SEQ ID NO: 73 - protein, 464 aa, Artificial sequence
  An artificially synthesized peptide sequence
QVQLVESGGGLVQPGHSLRLSCAASGFTFSNAWMHWVRQAPGKGLEWVAQIKDRGNNYAAYYAESVKGRFTISRDDSKNSIYLQMNSLKTEDTAVYYCRYVHYGSYFFASFYFGVDIWGQGTTVTVSSASTKGPSVFPLAPSSKSTSGGTAALGCLVKDYFPEPVTVSWNSGALTSGVHTFPAVLQSSGLYSLSSVVTVPSSSLGTQTYICNVNHKPSNTKVDKKVEPKSCDKTHTCPPCPAPEAAGGPSVFLFPPKPKDTLMISRTPEVTCVVVDVSHEDPEVKFNWYVDGVEVHNAKTKPREEQYASTYRVVSVLTVLHQDWLNGKEYKCKVSNKALPAPIEKTISKAKGQPREPQVYTLPPSRCELTKNQVSLSCAVKGFYPSDIAVEWESNGQPENNYKTTPPVLDSDGSFFLVSKLTVDKSRWQQGNVFSCSVMHEALHNHYTQKSLSLSPDYKDDDDK

SEQ ID NO: 74 - protein, 464 aa, Artificial sequence
  An artificially synthesized peptide sequence
QVQLVESGGGLVQPGRSLRLSCAASGFTFSNAWMHWVRQAPGKGLEWVAQIKDRGNNYNTYYAPSVKGRFTISRDDSKNSIYLQMNSLKTEDTAVYYCRYVHYGSYFFSGSSFGVDIWGQGTTVTVSSASTKGPSVFPLAPSSKSTSGGTAALGCLVKDYFPEPVTVSWNSGALTSGVHTFPAVLQSSGLYSLSSVVTVPSSSLGTQTYICNVNHKPSNTKVDKKVEPKSCDKTHTCPPCPAPEAAGGPSVFLFPPKPKDTLMISRTPEVTCVVVDVSHEDPEVKFNWYVDGVEVHNAKTKPREEQYASTYRVVSVLTVLHQDWLNGKEYKCKVSNKALPAPIEKTISKAKGQPREPQVYTLPPSRCELTKNQVSLSCAVKGFYPSDIAVEWESNGQPENNYKTTPPVLDSDGSFFLVSKLTVDKSRWQQGNVFSCSVMHEALHNHYTQKSLSLSPDYKDDDDK

SEQ ID NO: 75 - protein, 464 aa, Artificial sequence
  An artificially synthesized peptide sequence
QVQLVESGGGLVQPGRSLRLSCAASGFTFSNAWMHWVRQAPGKGLEWVAQIKDRGNNYNTYYAPSVKGRFTISRDDSKNSIYLQMNSLKTEDTAVYYCRYAHYGSYFFSGSSFGVDIWGQGTTVTVSSASTKGPSVFPLAPSSKSTSGGTAALGCLVKDYFPEPVTVSWNSGALTSGVHTFPAVLQSSGLYSLSSVVTVPSSSLGTQTYICNVNHKPSNTKVDKKVEPKSCDKTHTCPPCPAPEAAGGPSVFLFPPKPKDTLMISRTPEVTCVVVDVSHEDPEVKFNWYVDGVEVHNAKTKPREEQYASTYRVVSVLTVLHQDWLNGKEYKCKVSNKALPAPIEKTISKAKGQPREPQVYTLPPSRCELTKNQVSLSCAVKGFYPSDIAVEWESNGQPENNYKTTPPVLDSDGSFFLVSKLTVDKSRWQQGNVFSCSVMHEALHNHYTQKSLSLSPDYKDDDDK

SEQ ID NO: 76 - protein, 464 aa, Artificial sequence
  An artificially synthesized peptide sequence
QVQLVESGGGLVQPGRSLRLSCAASGFTFSNAWMHWVRQAPGKGLEWVAQIKDKGNQYATYYAESVKGRFTISRDDSKNSIYLQMNSLKTEDTAVYYCRYVHYGTYFFALPAFGVDIWGQGTTVTVSSASTKGPSVFPLAPSSKSTSGGTAALGCLVKDYFPEPVTVSWNSGALTSGVHTFPAVLQSSGLYSLSSVVTVPSSSLGTQTYICNVNHKPSNTKVDKKVEPKSCDKTHTCPPCPAPEAAGGPSVFLFPPKPKDTLMISRTPEVTCVVVDVSHEDPEVKFNWYVDGVEVHNAKTKPREEQYASTYRVVSVLTVLHQDWLNGKEYKCKVSNKALPAPIEKTISKAKGQPREPQVYTLPPSRCELTKNQVSLSCAVKGFYPSDIAVEWESNGQPENNYKTTPPVLDSDGSFFLVSKLTVDKSRWQQGNVFSCSVMHEALHNHYTQKSLSLSPDYKDDDDK

SEQ ID NO: 77 - protein, 464 aa, Artificial sequence
  An artificially synthesized peptide sequence
QVQLVESGGGLVQPGRSLRLSCAASGFTFSNAWMHWVRQAPGKGLEWVAQIKDKGNQYATYYAESVKGRYTISRDDSKNSIYLQMNSLKTEDTAVYYCRYVHYGTYFFALPAFGVDIWGQGTTVTVSSASTKGPSVFPLAPSSKSTSGGTAALGCLVKDYFPEPVTVSWNSGALTSGVHTFPAVLQSSGLYSLSSVVTVPSSSLGTQTYICNVNHKPSNTKVDKKVEPKSCDKTHTCPPCPAPEAAGGPSVFLFPPKPKDTLMISRTPEVTCVVVDVSHEDPEVKFNWYVDGVEVHNAKTKPREEQYASTYRVVSVLTVLHQDWLNGKEYKCKVSNKALPAPIEKTISKAKGQPREPQVYTLPPSRCELTKNQVSLSCAVKGFYPSDIAVEWESNGQPENNYKTTPPVLDSDGSFFLVSKLTVDKSRWQQGNVFSCSVMHEALHNHYTQKSLSLSPDYKDDDDK

SEQ ID NO: 78 - protein, 464 aa, Artificial sequence
  An artificially synthesized peptide sequence
QVQLVESGGGLVQPGRSLRLSCAASGFTFSNAWMHWVRQAPGKGLEWVAQIKDRGNNYAAYYAESVKGRFTISRDDSKNSIYLQMNSLKTEDTAVYYCRYVHYGSYFFASFYFGVDIWGQGTAVTVSSASTKGPSVFPLAPSSKSTSGGTAALGCLVKDYFPEPVTVSWNSGALTSGVHTFPAVLQSSGLYSLSSVVTVPSSSLGTQTYICNVNHKPSNTKVDKKVEPKSCDKTHTCPPCPAPEAAGGPSVFLFPPKPKDTLMISRTPEVTCVVVDVSHEDPEVKFNWYVDGVEVHNAKTKPREEQYASTYRVVSVLTVLHQDWLNGKEYKCKVSNKALPAPIEKTISKAKGQPREPQVYTLPPSRCELTKNQVSLSCAVKGFYPSDIAVEWESNGQPENNYKTTPPVLDSDGSFFLVSKLTVDKSRWQQGNVFSCSVMHEALHNHYTQKSLSLSPDYKDDDDK

SEQ ID NO: 79 - protein, 15 aa, Artificial sequence
  An artificially synthesized peptide sequence
GLNDIFEAQKIEWHE

SEQ ID NO: 80 - protein, 233 aa, Artificial sequence
  An artificially synthesized peptide sequence
CHPRLSLHRPALEDLLLGSEANLTCTLTGLRDASGVTFTWTPSSGKSAVQGPPERDLCGCYSVSSVLPGCAEPWNHGKTFTCTAAYPESKTPLTATLSKSGNTFRPEVHLLPPPSEELALNELVTLTCLARGFSPKDVLVRWLQGSQELPREKYLTWASRQEPSQGTTTFAVTSILRVAAEDWKKGDTFSCMVGHEALPLAFTQKTIDRLAGKGGGGSGLNDIFEAQKIEWHE

SEQ ID NO: 81 - protein, 641 aa, Human herpesvirus 4
MSDEGPGTGPGNGLGEKGDTSGPEGSGGSGPQRRGGDNHGRGRGRGRGRGGGRPGAPGGSGSGPRHRDGVRRPQKRPSCIGCKGTHGGTGAGAGAGGAGAGGAGAGGGAGAGGGAGGAGGAGGAGAGGGAGAGGGAGGAGGAGAGGGAGAGGGAGGAGAGGGAGGAGGAGAGGGAGAGGGAGGAGAGGGAGGAGGAGAGGGAGAGGAGGAGGAGAGGAGAGGGAGGAGGAGAGGAGAGGAGAGGAGAGGAGGAGAGGAGGAGAGGAGGAGAGGGAGGAGAGGGAGGAGAGGAGGAGAGGAGGAGAGGAGGAGAGGGAGAGGAGAGGGGRGRGGSGGRGRGGSGGRGRGGSGGRRGRGRERARGGSRERARGRGRGRGEKRPRSPSSQSSSSGSPPRRPPPGRRPFFHPVGEADYFEYHQEGGPDGEPDVPPGAIEQGPADDPGEGPSTGPRGQGDGGRRKKGGWFGKHRGQGGSNPKFENIAEGLRALLARSHVERTTDEGTWVAGVFVYGGSKTSLYNLRRGTALAIPQCRLTPLSRLPFGMAPGPGPQPGPLRESIVCYFMVFLQTHIFAEVLKDAIKDLVMTKPAPTCNIRVTVCSFDDGVDLPPWFPPMVEGAAAEGDDGDDGDEGGDGDEGEEGQE

SEQ ID NO: 82 - protein, 321 aa, Escherichia coli
MKDNTVPLKLIALLANGEFHSGEQLGETLGMSRAAINKHIQTLRDWGVDVFTVPGKGYSLPEPIQLLNAKQILGQLDGGSVAVLPVIDSTNQYLLDRIGELKSGDACIAEYQQAGRGRRGRKWFSPFGANLYLSMFWRLEQGPAAAIGLSLVIGIVMAEVLRKLGADKVRVKWPNDLYLQDRKLAGILVELTGKTGDAAQIVIGAGINMAMRRVEESVVNQGWITLQEAGINLDRNTLAAMLIRELRAALELFEQEGLAPYLSRWEKLDNFINRPVKLIIGDKEIFGISRGIDKQGALLLEQDGIIKPWMGGEISLRSAEK

SEQ ID NO: 83 - DNA, 549 bp, Homo sapiens
atggaacaggggaagggcctggctgtcctcatcctggctatcattcttcttcaaggtactttggcccagtcaatcaaaggaaaccacttggttaaggtgtatgactatcaagaagatggttcggtacttctgacttgtgatgcagaagccaaaaatatcacatggtttaaagatgggaagatgatcggcttcctaactgaagataaaaaaaaatggaatctgggaagtaatgccaaggaccctcgagggatgtatcagtgtaaaggatcacagaacaagtcaaaaccactccaagtgtattacagaatgtgtcagaactgcattgaactaaatgcagccaccatatctggctttctctttgctgaaatcgtcagcattttcgtccttgctgttggggtctacttcattgctggacaggatggagttcgccagtcgagagcttcagacaagcagactctgttgcccaatgaccagctctaccagcccctcaaggatcgagaagatgaccagtacagccaccttcaaggaaaccagttgaggaggaattga

SEQ ID NO: 84 - protein, 182 aa, Homo sapiens
MEQGKGLAVLILAIILLQGTLAQSIKGNHLVKVYDYQEDGSVLLTCDAEAKNITWFKDGKMIGFLTEDKKKWNLGSNAKDPRGMYQCKGSQNKSKPLQVYYRMCQNCIELNAATISGFLFAEIVSIFVLAVGVYFIAGQDGVRQSRASDKQTLLPNDQLYQPLKDREDDQYSHLQGNQLRRN

SEQ ID NO: 85 - DNA, 516 bp, Homo sapiens
atggaacatagcacgtttctctctggcctggtactggctacccttctctcgcaagtgagccccttcaagatacctatagaggaacttgaggacagagtgtttgtgaattgcaataccagcatcacatgggtagagggaacggtgggaacactgctctcagacattacaagactggacctgggaaaacgcatcctggacccacgaggaatatataggtgtaatgggacagatatatacaaggacaaagaatctaccgtgcaagttcattatcgaatgtgccagagctgtgtggagctggatccagccaccgtggctggcatcattgtcactgatgtcattgccactctgctccttgctttgggagtcttctgctttgctggacatgagactggaaggctgtctggggctgccgacacacaagctctgttgaggaatgaccaggtctatcagcccctccgagatcgagatgatgctcagtacagccaccttggaggaaactgggctcggaacaagtga

SEQ ID NO: 86 - protein, 171 aa, Homo sapiens
MEHSTFLSGLVLATLLSQVSPFKIPIEELEDRVFVNCNTSITWVEGTVGTLLSDITRLDLGKRILDPRGIYRCNGTDIYKDKESTVQVHYRMCQSCVELDPATVAGIIVTDVIATLLLALGVFCFAGHETGRLSGAADTQALLRNDQVYQPLRDRDDAQYSHLGGNWARNK

SEQ ID NO: 87 - DNA, 624 bp, Homo sapiens
atgcagtcgggcactcactggagagttctgggcctctgcctcttatcagttggcgtttgggggcaagatggtaatgaagaaatgggtggtattacacagacaccatataaagtctccatctctggaaccacagtaatattgacatgccctcagtatcctggatctgaaatactatggcaacacaatgataaaaacataggcggtgatgaggatgataaaaacataggcagtgatgaggatcacctgtcactgaaggaattttcagaattggagcaaagtggttattatgtctgctaccccagaggaagcaaaccagaagatgcgaacttttatctctacctgagggcaagagtgtgtgagaactgcatggagatggatgtgatgtcggtggccacaattgtcatagtggacatctgcatcactgggggcttgctgctgctggtttactactggagcaagaatagaaaggccaaggccaagcctgtgacacgaggagcgggtgctggcggcaggcaaaggggacaaaacaaggagaggccaccacctgttcccaacccagactatgagcccatccggaaaggccagcgggacctgtattctggcctgaatcagagacgcatctga

SEQ ID NO: 88 - protein, 207 aa, Homo sapiens
MQSGTHWRVLGLCLLSVGVWGQDGNEEMGGITQTPYKVSISGTTVILTCPQYPGSEILWQHNDKNIGGDEDDKNIGSDEDHLSLKEFSELEQSGYYVCYPRGSKPEDANFYLYLRARVCENCMEMDVMSVATIVIVDICITGGLLLLVYYWSKNRKAKAKPVTRGAGAGGRQRGQNKERPPPVPNPDYEPIRKGQRDLYSGLNQRRI

SEQ ID NO: 89 - protein, 8 aa, Artificial Sequence
  An artificially synthesized peptide sequence
DYKDDDDK

SEQ ID NO: 90 - protein, 6 aa, Artificial sequence
  An artificially synthesized peptide sequence
GGSGGS

SEQ ID NO: 91 - protein, 9 aa, Artificial sequence
  An artificially synthesized peptide sequence
GGSGGSGGS

SEQ ID NO: 92 - protein, 7 aa, Artificial sequence
  An artificially synthesized peptide sequence
GGSGGGS

SEQ ID NO: 93 - protein, 8 aa, Artificial sequence
  An artificially synthesized peptide sequence
GGGSGGGS